European Patent Application EP 4 253 532 A1, published October 4, 2023. Title: Isopropylmaleate synthase variant and a method of producing L-leucine using the same. Applicant: CJ CheilJedang Corporation. The sequence listing filed with the application follows.

SEQUENCE LISTING (55 sequences)

SEQ ID NO: 1 - protein, 616 aa, Unknown
  leuA(616 aa)
MSPNDAFISAPAKIETPVGPRNEGQPAWNKQRGSSMPVNRYMPFEVEVEDISLPDRTWPDKKITVAPQWCAVDLRDGNQALIDPMSPERKRRMFELLVQMGFKEIEVGFPSASQTDFDFVREIIEKGMIPDDVTIQVLVQAREHLIRRTFEACEGAKNVIVHFYNSTSILQRNVVFRMDKVQVKKLATDAAELIKTIAQDYPDTNWRWQYSPESFTGTEVEYAKEVVDAVVEVMDPTPENPMIINLPSTVEMITPNVYADSIEWMHRNLNRRDSIILSLHPHNDRGTGVGAAELGYMAGADRIEGCLFGNGERTGNVCLVTLALNMLTQGVDPQLDFTDIRQIRSTVEYCNQLRVPERHPYGGDLVFTAFSGSHQDAVNKGLDAMAAKVQPGASSTEVSWEQLRDTEWEVPYLPIDPKDVGRDYEAVIRVNSQSGKGGVAYIMKTDHGLQIPRSMQVEFSTVVQNVTDAEGGEVNSKAMWDIFATEYLERTAPVEQIALRVENAQTENEDASITAELIHNGKDVTVDGRGNGPLAAYANALEKLGIDVEIQEYNQHARTSGDDAEAAAYVLAEVNGRKVWGVGIAGSITYASLKAVTSAVNRALDVNHEAVLAGGV

SEQ ID NO: 2 - DNA, 1851 bp, Unknown
  leuA WT(1851 bp)
atgtctcctaacgatgcattcatctccgcacctgccaagatcgaaaccccagttgggcctcgcaacgaaggccagccagcatggaataagcagcgtggctcctcaatgccagttaaccgctacatgcctttcgaggttgaggtagaagatatttctctgccggaccgcacttggccagataaaaaaatcaccgttgcacctcagtggtgtgctgttgacctgcgtgacggcaaccaggctctgattgatccgatgtctcctgagcgtaagcgccgcatgtttgagctgctggttcagatgggcttcaaagaaatcgaggtcggtttcccttcagcttcccagactgattttgatttcgttcgtgagatcatcgaaaagggcatgatccctgacgatgtcaccattcaggttctggttcaggctcgtgagcacctgattcgccgtacttttgaagcttgcgaaggcgcaaaaaacgttatcgtgcacttctacaactccacctccatcctgcagcgcaacgtggtgttccgcatggacaaggtgcaggtgaagaagctggctaccgatgccgctgaactaatcaagaccatcgctcaggattacccagacaccaactggcgctggcagtactcccctgagtccttcaccggcactgaggttgagtacgccaaggaagttgtggacgcagttgttgaggtcatggatccaactcctgagaacccaatgatcatcaacctgccttccaccgttgagatgatcacccctaacgtttacgcagactccattgaatggatgcaccgcaatctaaaccgtcgtgattccattatcctgtccctgcacccgcacaatgaccgtggcaccggcgttggcgcagctgagctgggctacatggctggcgctgaccgcatcgaaggctgcctgttcggcaacggcgagcgcaccggcaacgtctgcctggtcaccctggcactgaacatgctgacccagggcgttgaccctcagctggacttcaccgatatacgccagatccgcagcaccgttgaatactgcaaccagctgcgcgttcctgagcgccacccatacggcggtgacctggtcttcaccgctttctccggttcccaccaggacgctgtgaacaagggtctggacgccatggctgccaaggttcagccaggtgctagctccactgaagtttcttgggagcagctgcgcgacaccgaatgggaggttccttacctgcctatcgatccaaaggatgtcggtcgcgactacgaggctgttatccgcgtgaactcccagtccggcaagggcggcgttgcttacatcatgaagaccgatcacggtctgcagatccctcgctccatgcaggttgagttctccaccgttgtccagaacgtcaccgacgctgagggcggcgaggtcaactccaaggcaatgtgggatatcttcgccaccgagtacctggagcgcaccgcaccagttgagcagatcgcgctgcgcgtcgagaacgctcagaccgaaaacgaggatgcatccatcaccgccgagctcatccacaacggcaaggacgtcaccgtcgatggccgcggcaacggcccactggccgcttacgccaacgcgctggagaagctgggcatcgacgttgagatccaggaatacaaccagcacgcccgcacctcgggcgacgatgcagaagcagccgcctacgtgctggctgaggtcaacggccgcaaggtctggggcgtcggcatcgctggctccatcacctacgcttcgctgaaggcagtgacctccgccgtaaaccgcgcgctggacgtcaaccacgaggcagtcctggctggcggcgtttaa

SEQ ID NO: 3 - DNA, 21 bp, Artificial Sequence
  Primer 1
tatgcttcaccacatgacttc

SEQ ID NO: 4 - DNA, 23 bp, Artificial Sequence
  Primer 2
aaatcatttgagaaaactcgagg

SEQ ID NO: 5 - protein, 581 aa, Unknown
  leuA(581 aa)
MPVNRYMPFEVEVEDISLPDRTWPDKKITVAPQWCAVDLRDGNQALIDPMSPERKRRMFELLVQMGFKEIEVGFPSASQTDFDFVREIIEKGMIPDDVTIQVLVQAREHLIRRTFEACEGAKNVIVHFYNSTSILQRNVVFRMDKVQVKKLATDAAELIKTIAQDYPDTNWRWQYSPESFTGTEVEYAKEVVDAVVEVMDPTPENPMIINLPSTVEMITPNVYADSIEWMHRNLNRRDSIILSLHPHNDRGTGVGAAELGYMAGADRIEGCLFGNGERTGNVCLVTLALNMLTQGVDPQLDFTDIRQIRSTVEYCNQLRVPERHPYGGDLVFTAFSGSHQDAVNKGLDAMAAKVQPGASSTEVSWEQLRDTEWEVPYLPIDPKDVGRDYEAVIRVNSQSGKGGVAYIMKTDHGLQIPRSMQVEFSTVVQNVTDAEGGEVNSKAMWDIFATEYLERTAPVEQIALRVENAQTENEDASITAELIHNGKDVTVDGRGNGPLAAYANALEKLGIDVEIQEYNQHARTSGDDAEAAAYVLAEVNGRKVWGVGIAGSITYASLKAVTSAVNRALDVNHEAVLAGGV

SEQ ID NO: 6 - protein, 616 aa, Artificial Sequence
  L138G
MSPNDAFISAPAKIETPVGPRNEGQPAWNKQRGSSMPVNRYMPFEVEVEDISLPDRTWPDKKITVAPQWCAVDLRDGNQALIDPMSPERKRRMFELLVQMGFKEIEVGFPSASQTDFDFVREIIEKGMIPDDVTIQVGVQAREHLIRRTFEACEGAKNVIVHFYNSTSILQRNVVFRMDKVQVKKLATDAAELIKTIAQDYPDTNWRWQYSPESFTGTEVEYAKEVVDAVVEVMDPTPENPMIINLPSTVEMITPNVYADSIEWMHRNLNRRDSIILSLHPHNDRGTGVGAAELGYMAGADRIEGCLFGNGERTGNVCLVTLALNMLTQGVDPQLDFTDIRQIRSTVEYCNQLRVPERHPYGGDLVFTAFSGSHQDAVNKGLDAMAAKVQPGASSTEVSWEQLRDTEWEVPYLPIDPKDVGRDYEAVIRVNSQSGKGGVAYIMKTDHGLQIPRSMQVEFSTVVQNVTDAEGGEVNSKAMWDIFATEYLERTAPVEQIALRVENAQTENEDASITAELIHNGKDVTVDGRGNGPLAAYANALEKLGIDVEIQEYNQHARTSGDDAEAAAYVLAEVNGRKVWGVGIAGSITYASLKAVTSAVNRALDVNHEAVLAGGV

SEQ ID NO: 7 - DNA, 1851 bp, Artificial Sequence
  L138G
atgtctcctaacgatgcattcatctccgcacctgccaagatcgaaaccccagttgggcctcgcaatgaaggccagccagcatggaataagcagcgtggctcctcaatgccagttaaccgctacatgcctttcgaggttgaggtagaagatatttctctgccggaccgcacttggccagataaaaaaatcaccgttgcacctcagtggtgtgctgttgacctgcgtgacggcaaccaggctctgattgatccgatgtctcctgagcgtaagcgccgcatgtttgagctgctggttcagatgggattcaaggaaatcgaggtcggtttcccttcagcttcccagactgattttgatttcgttcgtgagatcatcgaaaaggacatgatccctgacgatgtcaccattcaggttggggttcaggctcgtgagcacctgattcgccgtacttttgaagcttgcgaaggcgcaaaaaacgttatcgtgcacttctacaactcaacctccatcctgcagcgcaacgtggtgttccgcatggacaaggtgcaggtgaagaagctggctaccgatgccgctgaactgatcaagaccgtcgctcaggattacccagacaccaactggcgctggcagtactcccctgagtccttcaccggcactgaggttgagtacgccaaggaagttgtggacgcagttgttgaggtcatggatccaactcctgagaacccaatgatcatcaacctgccttccaccgttgagatgatcacccctaacgtttacgcagactccattgaatggatgcaccgcaatctaaaccgtcgtgattccattatcctgtccctgcacccgcacaatgaccgtggcaccggcgttggcgcagctgagctgggctacatggctggcgctgaccgcatcgaaggctgcctgttcggcaacggcgagcgcaccggcaacgtctgcctggtcaccctggcactgaacatgctgacccagggcgttgaccctcagctggacttcaccgatatacgccagatccgcagcaccgttgaatactgcaaccagctgcgcgttcctgagcgccacccatacggcggcgacctggtcttcaccgctttctccggttcccaccaggacgctgtgaacaagggtctggacgccatggctgccaaggttcagccaggtgctagctccactgaagtttcttgggagcagctgcgcgacaccgaatgggaggttccttacctgcctatcgatccaaaggatgtcggtcgcgactacgaggctgttatccgcgtgaactcccagtccggcaagggcggcgttgcttacatcatgaagaccgatcacggtctgcagatccctcgctccatgcaggttgagttctccaccgttgtccagaacgtcaccgacgctgagggcggcgaggtcaactccaaggcaatgtgggatatcttcgccaccgagtacctggagcgcaccgcaccagttgagcagatcgcgctgcgcgtcgagaacgctcagaccgaaaacgaggatgcatccatcaccgccgagctcatccacaacggcaaggacgtcaccgtcgatggccacggcaacggcccactggctgcttacgccaacgcgctggagaagctgggcatcgacgttgagatccaggaatacaaccagcacgcccgcacctcgggcgacgatgcagaagcagccgcctacgtgctggctgaggtcaacggccgcaaggtctggggcgtcggcatcgctggctccatcacctacgcttcgctgaaggcagtgacctccgccgtaaaccgcgcgctggacgtcaaccacgaggcagtcctggctggcggcgtttaa

SEQ ID NO: 8 - protein, 616 aa, Artificial Sequence
  H162E
MSPNDAFISAPAKIETPVGPRNEGQPAWNKQRGSSMPVNRYMPFEVEVEDISLPDRTWPDKKITVAPQWCAVDLRDGNQALIDPMSPERKRRMFELLVQMGFKEIEVGFPSASQTDFDFVREIIEKGMIPDDVTIQVGVQAREHLIRRTFEACEGAKNVIVEFYNSTSILQRNVVFRMDKVQVKKLATDAAELIKTIAQDYPDTNWRWQYSPESFTGTEVEYAKEVVDAVVEVMDPTPENPMIINLPSTVEMITPNVYADSIEWMHRNLNRRDSIILSLHPHNDRGTGVGAAELGYMAGADRIEGCLFGNGERTGNVCLVTLALNMLTQGVDPQLDFTDIRQIRSTVEYCNQLRVPERHPYGGDLVFTAFSGSHQDAVNKGLDAMAAKVQPGASSTEVSWEQLRDTEWEVPYLPIDPKDVGRDYEAVIRVNSQSGKGGVAYIMKTDHGLQIPRSMQVEFSTVVQNVTDAEGGEVNSKAMWDIFATEYLERTAPVEQIALRVENAQTENEDASITAELIHNGKDVTVDGRGNGPLAAYANALEKLGIDVEIQEYNQHARTSGDDAEAAAYVLAEVNGRKVWGVGIAGSITYASLKAVTSAVNRALDVNHEAVLAGGV

SEQ ID NO: 9 - DNA, 1851 bp, Artificial Sequence
  H162E
atgtctcctaacgatgcattcatctccgcacctgccaagatcgaaaccccagttgggcctcgcaatgaaggccagccagcatggaataagcagcgtggctcctcaatgccagttaaccgctacatgcctttcgaggttgaggtagaagatatttctctgccggaccgcacttggccagataaaaaaatcaccgttgcacctcagtggtgtgctgttgacctgcgtgacggcaaccaggctctgattgatccgatgtctcctgagcgtaagcgccgcatgtttgagctgctggttcagatgggattcaaggaaatcgaggtcggtttcccttcagcttcccagactgattttgatttcgttcgtgagatcatcgaaaaggacatgatccctgacgatgtcaccattcaggttctggttcaggctcgtgagcacctgattcgccgtacttttgaagcttgcgaaggcgcaaaaaacgttatcgtggagttctacaactcaacctccatcctgcagcgcaacgtggtgttccgcatggacaaggtgcaggtgaagaagctggctaccgatgccgctgaactgatcaagaccgtcgctcaggattacccagacaccaactggcgctggcagtactcccctgagtccttcaccggcactgaggttgagtacgccaaggaagttgtggacgcagttgttgaggtcatggatccaactcctgagaacccaatgatcatcaacctgccttccaccgttgagatgatcacccctaacgtttacgcagactccattgaatggatgcaccgcaatctaaaccgtcgtgattccattatcctgtccctgcacccgcacaatgaccgtggcaccggcgttggcgcagctgagctgggctacatggctggcgctgaccgcatcgaaggctgcctgttcggcaacggcgagcgcaccggcaacgtctgcctggtcaccctggcactgaacatgctgacccagggcgttgaccctcagctggacttcaccgatatacgccagatccgcagcaccgttgaatactgcaaccagctgcgcgttcctgagcgccacccatacggcggcgacctggtcttcaccgctttctccggttcccaccaggacgctgtgaacaagggtctggacgccatggctgccaaggttcagccaggtgctagctccactgaagtttcttgggagcagctgcgcgacaccgaatgggaggttccttacctgcctatcgatccaaaggatgtcggtcgcgactacgaggctgttatccgcgtgaactcccagtccggcaagggcggcgttgcttacatcatgaagaccgatcacggtctgcagatccctcgctccatgcaggttgagttctccaccgttgtccagaacgtcaccgacgctgagggcggcgaggtcaactccaaggcaatgtgggatatcttcgccaccgagtacctggagcgcaccgcaccagttgagcagatcgcgctgcgcgtcgagaacgctcagaccgaaaacgaggatgcatccatcaccgccgagctcatccacaacggcaaggacgtcaccgtcgatggccacggcaacggcccactggctgcttacgccaacgcgctggagaagctgggcatcgacgttgagatccaggaatacaaccagcacgcccgcacctcgggcgacgatgcagaagcagccgcctacgtgctggctgaggtcaacggccgcaaggtctggggcgtcggcatcgctggctccatcacctacgcttcgctgaaggcagtgacctccgccgtaaaccgcgcgctggacgtcaaccacgaggcagtcctggctggcggcgtttaa

SEQ ID NO: 10 - protein, 616 aa, Artificial Sequence
  S211L
MSPNDAFISAPAKIETPVGPRNEGQPAWNKQRGSSMPVNRYMPFEVEVEDISLPDRTWPDKKITVAPQWCAVDLRDGNQALIDPMSPERKRRMFELLVQMGFKEIEVGFPSASQTDFDFVREIIEKGMIPDDVTIQVGVQAREHLIRRTFEACEGAKNVIVEFYNSTSILQRNVVFRMDKVQVKKLATDAAELIKTIAQDYPDTNWRWQYLPESFTGTEVEYAKEVVDAVVEVMDPTPENPMIINLPSTVEMITPNVYADSIEWMHRNLNRRDSIILSLHPHNDRGTGVGAAELGYMAGADRIEGCLFGNGERTGNVCLVTLALNMLTQGVDPQLDFTDIRQIRSTVEYCNQLRVPERHPYGGDLVFTAFSGSHQDAVNKGLDAMAAKVQPGASSTEVSWEQLRDTEWEVPYLPIDPKDVGRDYEAVIRVNSQSGKGGVAYIMKTDHGLQIPRSMQVEFSTVVQNVTDAEGGEVNSKAMWDIFATEYLERTAPVEQIALRVENAQTENEDASITAELIHNGKDVTVDGRGNGPLAAYANALEKLGIDVEIQEYNQHARTSGDDAEAAAYVLAEVNGRKVWGVGIAGSITYASLKAVTSAVNRALDVNHEAVLAGGV

SEQ ID NO: 11 - DNA, 1851 bp, Artificial Sequence
  S211L
atgtctcctaacgatgcattcatctccgcacctgccaagatcgaaaccccagttgggcctcgcaatgaaggccagccagcatggaataagcagcgtggctcctcaatgccagttaaccgctacatgcctttcgaggttgaggtagaagatatttctctgccggaccgcacttggccagataaaaaaatcaccgttgcacctcagtggtgtgctgttgacctgcgtgacggcaaccaggctctgattgatccgatgtctcctgagcgtaagcgccgcatgtttgagctgctggttcagatgggattcaaggaaatcgaggtcggtttcccttcagcttcccagactgattttgatttcgttcgtgagatcatcgaaaaggacatgatccctgacgatgtcaccattcaggttctggttcaggctcgtgagcacctgattcgccgtacttttgaagcttgcgaaggcgcaaaaaacgttatcgtgcacttctacaactcaacctccatcctgcagcgcaacgtggtgttccgcatggacaaggtgcaggtgaagaagctggctaccgatgccgctgaactgatcaagaccgtcgctcaggattacccagacaccaactggcgctggcagtaccttcctgagtccttcaccggcactgaggttgagtacgccaaggaagttgtggacgcagttgttgaggtcatggatccaactcctgagaacccaatgatcatcaacctgccttccaccgttgagatgatcacccctaacgtttacgcagactccattgaatggatgcaccgcaatctaaaccgtcgtgattccattatcctgtccctgcacccgcacaatgaccgtggcaccggcgttggcgcagctgagctgggctacatggctggcgctgaccgcatcgaaggctgcctgttcggcaacggcgagcgcaccggcaacgtctgcctggtcaccctggcactgaacatgctgacccagggcgttgaccctcagctggacttcaccgatatacgccagatccgcagcaccgttgaatactgcaaccagctgcgcgttcctgagcgccacccatacggcggcgacctggtcttcaccgctttctccggttcccaccaggacgctgtgaacaagggtctggacgccatggctgccaaggttcagccaggtgctagctccactgaagtttcttgggagcagctgcgcgacaccgaatgggaggttccttacctgcctatcgatccaaaggatgtcggtcgcgactacgaggctgttatccgcgtgaactcccagtccggcaagggcggcgttgcttacatcatgaagaccgatcacggtctgcagatccctcgctccatgcaggttgagttctccaccgttgtccagaacgtcaccgacgctgagggcggcgaggtcaactccaaggcaatgtgggatatcttcgccaccgagtacctggagcgcaccgcaccagttgagcagatcgcgctgcgcgtcgagaacgctcagaccgaaaacgaggatgcatccatcaccgccgagctcatccacaacggcaaggacgtcaccgtcgatggccacggcaacggcccactggctgcttacgccaacgcgctggagaagctgggcatcgacgttgagatccaggaatacaaccagcacgcccgcacctcgggcgacgatgcagaagcagccgcctacgtgctggctgaggtcaacggccgcaaggtctggggcgtcggcatcgctggctccatcacctacgcttcgctgaaggcagtgacctccgccgtaaaccgcgcgctggacgtcaaccacgaggcagtcctggctggcggcgtttaa

SEQ ID NO: 12 - protein, 616 aa, Artificial Sequence
  I588P
MSPNDAFISAPAKIETPVGPRNEGQPAWNKQRGSSMPVNRYMPFEVEVEDISLPDRTWPDKKITVAPQWCAVDLRDGNQALIDPMSPERKRRMFELLVQMGFKEIEVGFPSASQTDFDFVREIIEKGMIPDDVTIQVGVQAREHLIRRTFEACEGAKNVIVEFYNSTSILQRNVVFRMDKVQVKKLATDAAELIKTIAQDYPDTNWRWQYLPESFTGTEVEYAKEVVDAVVEVMDPTPENPMIISLPSTVEMITPNVYADSIEWMHRNLNRRDSIILSLHPHNDRGTGVGAAELGYMAGADRIEGCLFGNGERTGNVCLVTLALNMLTQGVDPQLDFTDIRQIRSTVEYCNQLRVPERHPYGGDLVFTAFSGSHQDAVNKGLDAMAAKVQPGASSTEVSWEQLRDTEWEVPYLPIDPKDVGRDYEAVIRVNSQSGKGGVAYIMKTDHGLQIPRSMQVEFSTVVQNVTDAEGGEVNSKAMWDIFATEYLERTAPVEQIALRVENAQTENEDASITAELIHNGKDVTVDGRGNGPLAAYANALEKLGIDVEIQEYNQHARTSGDDAEAAAYVLAEVNGRKVWGVGIAGSPTYASLKAVTSAVNRALDVNHEAVLAGGV

SEQ ID NO: 13 - DNA, 1851 bp, Artificial Sequence
  I588P
atgtctcctaacgatgcattcatctccgcacctgccaagatcgaaaccccagttgggcctcgcaatgaaggccagccagcatggaataagcagcgtggctcctcaatgccagttaaccgctacatgcctttcgaggttgaggtagaagatatttctctgccggaccgcacttggccagataaaaaaatcaccgttgcacctcagtggtgtgctgttgacctgcgtgacggcaaccaggctctgattgatccgatgtctcctgagcgtaagcgccgcatgtttgagctgctggttcagatgggattcaaggaaatcgaggtcggtttcccttcagcttcccagactgattttgatttcgttcgtgagatcatcgaaaaggacatgatccctgacgatgtcaccattcaggttctggttcaggctcgtgagcacctgattcgccgtacttttgaagcttgcgaaggcgcaaaaaacgttatcgtgcacttctacaactcaacctccatcctgcagcgcaacgtggtgttccgcatggacaaggtgcaggtgaagaagctggctaccgatgccgctgaactgatcaagaccgtcgctcaggattacccagacaccaactggcgctggcagtactcccctgagtccttcaccggcactgaggttgagtacgccaaggaagttgtggacgcagttgttgaggtcatggatccaactcctgagaacccaatgatcatcaacctgccttccaccgttgagatgatcacccctaacgtttacgcagactccattgaatggatgcaccgcaatctaaaccgtcgtgattccattatcctgtccctgcacccgcacaatgaccgtggcaccggcgttggcgcagctgagctgggctacatggctggcgctgaccgcatcgaaggctgcctgttcggcaacggcgagcgcaccggcaacgtctgcctggtcaccctggcactgaacatgctgacccagggcgttgaccctcagctggacttcaccgatatacgccagatccgcagcaccgttgaatactgcaaccagctgcgcgttcctgagcgccacccatacggcggcgacctggtcttcaccgctttctccggttcccaccaggacgctgtgaacaagggtctggacgccatggctgccaaggttcagccaggtgctagctccactgaagtttcttgggagcagctgcgcgacaccgaatgggaggttccttacctgcctatcgatccaaaggatgtcggtcgcgactacgaggctgttatccgcgtgaactcccagtccggcaagggcggcgttgcttacatcatgaagaccgatcacggtctgcagatccctcgctccatgcaggttgagttctccaccgttgtccagaacgtcaccgacgctgagggcggcgaggtcaactccaaggcaatgtgggatatcttcgccaccgagtacctggagcgcaccgcaccagttgagcagatcgcgctgcgcgtcgagaacgctcagaccgaaaacgaggatgcatccatcaccgccgagctcatccacaacggcaaggacgtcaccgtcgatggccacggcaacggcccactggctgcttacgccaacgcgctggagaagctgggcatcgacgttgagatccaggaatacaaccagcacgcccgcacctcgggcgacgatgcagaagcagccgcctacgtgctggctgaggtcaacggccgcaaggtctggggcgtcggcatcgctggctcccccacctacgcttcgctgaaggcagtgacctccgccgtaaaccgcgcgctggacgtcaaccacgaggcagtcctggctggcggcgtttaa

SEQ ID NO: 14 - protein, 616 aa, Artificial Sequence
  N245S
MSPNDAFISAPAKIETPVGPRNEGQPAWNKQRGSSMPVNRYMPFEVEVEDISLPDRTWPDKKITVAPQWCAVDLRDGNQALIDPMSPERKRRMFELLVQMGFKEIEVGFPSASQTDFDFVREIIEKGMIPDDVTIQVGVQAREHLIRRTFEACEGAKNVIVEFYNSTSILQRNVVFRMDKVQVKKLATDAAELIKTIAQDYPDTNWRWQYLPESFTGTEVEYAKEVVDAVVEVMDPTPENPMIISLPSTVEMITPNVYADSIEWMHRNLNRRDSIILSLHPHNDRGTGVGAAELGYMAGADRIEGCLFGNGERTGNVCLVTLALNMLTQGVDPQLDFTDIRQIRSTVEYCNQLRVPERHPYGGDLVFTAFSGSHQDAVNKGLDAMAAKVQPGASSTEVSWEQLRDTEWEVPYLPIDPKDVGRDYEAVIRVNSQSGKGGVAYIMKTDHGLQIPRSMQVEFSTVVQNVTDAEGGEVNSKAMWDIFATEYLERTAPVEQIALRVENAQTENEDASITAELIHNGKDVTVDGRGNGPLAAYANALEKLGIDVEIQEYNQHARTSGDDAEAAAYVLAEVNGRKVWGVGIAGSITYASLKAVTSAVNRALDVNHEAVLAGGV

SEQ ID NO: 15 - DNA, 1851 bp, Artificial Sequence
  N245S
atgtctcctaacgatgcattcatctccgcacctgccaagatcgaaaccccagttgggcctcgcaatgaaggccagccagcatggaataagcagcgtggctcctcaatgccagttaaccgctacatgcctttcgaggttgaggtagaagatatttctctgccggaccgcacttggccagataaaaaaatcaccgttgcacctcagtggtgtgctgttgacctgcgtgacggcaaccaggctctgattgatccgatgtctcctgagcgtaagcgccgcatgtttgagctgctggttcagatgggattcaaggaaatcgaggtcggtttcccttcagcttcccagactgattttgatttcgttcgtgagatcatcgaaaaggacatgatccctgacgatgtcaccattcaggttctggttcaggctcgtgagcacctgattcgccgtacttttgaagcttgcgaaggcgcaaaaaacgttatcgtgcacttctacaactcaacctccatcctgcagcgcaacgtggtgttccgcatggacaaggtgcaggtgaagaagctggctaccgatgccgctgaactgatcaagaccgtcgctcaggattacccagacaccaactggcgctggcagtactcccctgagtccttcaccggcactgaggttgagtacgccaaggaagttgtggacgcagttgttgaggtcatggatccaactcctgagaacccaatgatcatctccctgccttccaccgttgagatgatcacccctaacgtttacgcagactccattgaatggatgcaccgcaatctaaaccgtcgtgattccattatcctgtccctgcacccgcacaatgaccgtggcaccggcgttggcgcagctgagctgggctacatggctggcgctgaccgcatcgaaggctgcctgttcggcaacggcgagcgcaccggcaacgtctgcctggtcaccctggcactgaacatgctgacccagggcgttgaccctcagctggacttcaccgatatacgccagatccgcagcaccgttgaatactgcaaccagctgcgcgttcctgagcgccacccatacggcggcgacctggtcttcaccgctttctccggttcccaccaggacgctgtgaacaagggtctggacgccatggctgccaaggttcagccaggtgctagctccactgaagtttcttgggagcagctgcgcgacaccgaatgggaggttccttacctgcctatcgatccaaaggatgtcggtcgcgactacgaggctgttatccgcgtgaactcccagtccggcaagggcggcgttgcttacatcatgaagaccgatcacggtctgcagatccctcgctccatgcaggttgagttctccaccgttgtccagaacgtcaccgacgctgagggcggcgaggtcaactccaaggcaatgtgggatatcttcgccaccgagtacctggagcgcaccgcaccagttgagcagatcgcgctgcgcgtcgagaacgctcagaccgaaaacgaggatgcatccatcaccgccgagctcatccacaacggcaaggacgtcaccgtcgatggccacggcaacggcccactggctgcttacgccaacgcgctggagaagctgggcatcgacgttgagatccaggaatacaaccagcacgcccgcacctcgggcgacgatgcagaagcagccgcctacgtgctggctgaggtcaacggccgcaaggtctggggcgtcggcatcgctggctccatcacctacgcttcgctgaaggcagtgacctccgccgtaaaccgcgcgctggacgtcaaccacgaggcagtcctggctggcggcgtttaa

SEQ ID NO: 16 - DNA, 42 bp, Artificial Sequence
  Primer 3
ggtcgactctagaggatcccctatgcttcaccacatgacttc

SEQ ID NO: 17 - DNA, 42 bp, Artificial Sequence
  Primer 4
caggtgctcacgagcctgaaccccaacctgaatggtgacatc

SEQ ID NO: 18 - DNA, 39 bp, Artificial Sequence
  Primer 5
gacgatgtcaccattcaggttggggttcaggctcgtgag

SEQ ID NO: 19 - DNA, 45 bp, Artificial Sequence
  Primer 6
gtgaattcgagctcggtacccaaatcatttgagaaaactcgaggc

SEQ ID NO: 20 - DNA, 43 bp, Artificial Sequence
  Primer 7
gatggaggttgagttgtagaactccacgataacgttttttgcg

SEQ ID NO: 21 - DNA, 42 bp, Artificial Sequence
  Primer 8
ggcgcaaaaaacgttatcgtggagttctacaactcaacctcc

SEQ ID NO: 22 - DNA, 38 bp, Artificial Sequence
  Primer 9
agtgccggtgaaggactcaggaaggtactgccagcgcc

SEQ ID NO: 23 - DNA, 39 bp, Artificial Sequence
  Primer 10
accaactggcgctggcagtaccttcctgagtccttcacc

SEQ ID NO: 24 - DNA, 42 bp, Artificial Sequence
  Primer 11
catctcaacggtggaacacagggagatgatcattgggttctc

SEQ ID NO: 25 - DNA, 37 bp, Artificial Sequence
  Primer 12
cctgagaacccaatgatcatctccctgtgttccaccg

SEQ ID NO: 26 - DNA, 38 bp, Artificial Sequence
  Primer 13
tgccttcagcgaagcgtaggtgggggagccagcgatgc

SEQ ID NO: 27 - DNA, 39 bp, Artificial Sequence
  Primer 14
ggcgtcggcatcgctggctcccccacctacgcttcgctg

SEQ ID NO: 28 - DNA, 22 bp, Artificial Sequence
  Primer 15
aacacgaccggcatcccgtcgc

SEQ ID NO: 29 - DNA, 23 bp, Artificial Sequence
  Primer 16
aaatcatttgagaaaactcgagg

SEQ ID NO: 30 - DNA, 19 bp, Artificial Sequence
  Primer 23
gtcacccgatcgtctgaag

SEQ ID NO: 31 - DNA, 18 bp, Artificial Sequence
  Primer 24
gtcttaaaaccggttgat

SEQ ID NO: 32 - DNA, 42 bp, Artificial Sequence
  gltA M312I Up F
gtgaattcgagctcggtacccgcgggaatcctgcgttaccgc

SEQ ID NO: 33 - DNA, 42 bp, Artificial Sequence
  gltA M312I Up R
tgtaaacgcggtgtccgaagccgatgaggcggacgccgtctt

SEQ ID NO: 34 - DNA, 42 bp, Artificial Sequence
  gltA M312I Down F
aagacggcgtccgcctcatcggcttcggacaccgcgtttaca

SEQ ID NO: 35 - DNA, 42 bp, Artificial Sequence
  gltA M312I Down R
ggtcgactctagaggatccccttagcgctcctcgcgaggaac

SEQ ID NO: 36 - DNA, 19 bp, Artificial Sequence
  Primer 25
caatgctggctgcgtacgc

SEQ ID NO: 37 - DNA, 20 bp, Artificial Sequence
  Primer 26
ctcctcgcgaggaaccaact

SEQ ID NO: 38 - protein, 616 aa, Artificial Sequence
  L138G, P247C, R558H, G561D
MSPNDAFISAPAKIETPVGPRNEGQPAWNKQRGSSMPVNRYMPFEVEVEDISLPDRTWPDKKITVAPQWCAVDLRDGNQALIDPMSPERKRRMFELLVQMGFKEIEVGFPSASQTDFDFVREIIEKGMIPDDVTIQVGVQAREHLIRRTFEACEGAKNVIVHFYNSTSILQRNVVFRMDKVQVKKLATDAAELIKTIAQDYPDTNWRWQYSPESFTGTEVEYAKEVVDAVVEVMDPTPENPMIINLCSTVEMITPNVYADSIEWMHRNLNRRDSIILSLHPHNDRGTGVGAAELGYMAGADRIEGCLFGNGERTGNVCLVTLALNMLTQGVDPQLDFTDIRQIRSTVEYCNQLRVPERHPYGGDLVFTAFSGSHQDAVNKGLDAMAAKVQPGASSTEVSWEQLRDTEWEVPYLPIDPKDVGRDYEAVIRVNSQSGKGGVAYIMKTDHGLQIPRSMQVEFSTVVQNVTDAEGGEVNSKAMWDIFATEYLERTAPVEQIALRVENAQTENEDASITAELIHNGKDVTVDGRGNGPLAAYANALEKLGIDVEIQEYNQHAHTSDDDAEAAAYVLAEVNGRKVWGVGIAGSITYASLKAVTSAVNRALDVNHEAVLAGGV

SEQ ID NO: 39 - DNA, 1851 bp, Artificial Sequence
  L138G, P247C, R558H, G561D
atgtctcctaacgatgcattcatctccgcacctgccaagatcgaaaccccagttgggcctcgcaatgaaggccagccagcatggaataagcagcgtggctcctcaatgccagttaaccgctacatgcctttcgaggttgaggtagaagatatttctctgccggaccgcacttggccagataaaaaaatcaccgttgcacctcagtggtgtgctgttgacctgcgtgacggcaaccaggctctgattgatccgatgtctcctgagcgtaagcgccgcatgtttgagctgctggttcagatgggattcaaggaaatcgaggtcggtttcccttcagcttcccagactgattttgatttcgttcgtgagatcatcgaaaaggacatgatccctgacgatgtcaccattcaggttggggttcaggctcgtgagcacctgattcgccgtacttttgaagcttgcgaaggcgcaaaaaacgttatcgtgcacttctacaactcaacctccatcctgcagcgcaacgtggtgttccgcatggacaaggtgcaggtgaagaagctggctaccgatgccgctgaactgatcaagaccgtcgctcaggattacccagacaccaactggcgctggcagtactcccctgagtccttcaccggcactgaggttgagtacgccaaggaagttgtggacgcagttgttgaggtcatggatccaactcctgagaacccaatgatcatcaacctgtgttccaccgttgagatgatcacccctaacgtttacgcagactccattgaatggatgcaccgcaatctaaaccgtcgtgattccattatcctgtccctgcacccgcacaatgaccgtggcaccggcgttggcgcagctgagctgggctacatggctggcgctgaccgcatcgaaggctgcctgttcggcaacggcgagcgcaccggcaacgtctgcctggtcaccctggcactgaacatgctgacccagggcgttgaccctcagctggacttcaccgatatacgccagatccgcagcaccgttgaatactgcaaccagctgcgcgttcctgagcgccacccatacggcggcgacctggtcttcaccgctttctccggttcccaccaggacgctgtgaacaagggtctggacgccatggctgccaaggttcagccaggtgctagctccactgaagtttcttgggagcagctgcgcgacaccgaatgggaggttccttacctgcctatcgatccaaaggatgtcggtcgcgactacgaggctgttatccgcgtgaactcccagtccggcaagggcggcgttgcttacatcatgaagaccgatcacggtctgcagatccctcgctccatgcaggttgagttctccaccgttgtccagaacgtcaccgacgctgagggcggcgaggtcaactccaaggcaatgtgggatatcttcgccaccgagtacctggagcgcaccgcaccagttgagcagatcgcgctgcgcgtcgagaacgctcagaccgaaaacgaggatgcatccatcaccgccgagctcatccacaacggcaaggacgtcaccgtcgatggccacggcaacggcccactggctgcttacgccaacgcgctggagaagctgggcatcgacgttgagatccaggaatacaaccagcacgcccacacctcggatgacgatgcagaagcagccgcctacgtgctggctgaggtcaacggccgcaaggtctggggcgtcggcatcgctggctccatcacctacgcttcgctgaaggcagtgacctccgccgtaaaccgcgcgctggacgtcaaccacgaggcagtcctggctggcggcgtttaa

SEQ ID NO: 40 - protein, 616 aa, Artificial Sequence
  H162E, P247C, R558H, G561D
MSPNDAFISAPAKIETPVGPRNEGQPAWNKQRGSSMPVNRYMPFEVEVEDISLPDRTWPDKKITVAPQWCAVDLRDGNQALIDPMSPERKRRMFELLVQMGFKEIEVGFPSASQTDFDFVREIIEKGMIPDDVTIQVLVQAREHLIRRTFEACEGAKNVIVEFYNSTSILQRNVVFRMDKVQVKKLATDAAELIKTIAQDYPDTNWRWQYSPESFTGTEVEYAKEVVDAVVEVMDPTPENPMIINLCSTVEMITPNVYADSIEWMHRNLNRRDSIILSLHPHNDRGTGVGAAELGYMAGADRIEGCLFGNGERTGNVCLVTLALNMLTQGVDPQLDFTDIRQIRSTVEYCNQLRVPERHPYGGDLVFTAFSGSHQDAVNKGLDAMAAKVQPGASSTEVSWEQLRDTEWEVPYLPIDPKDVGRDYEAVIRVNSQSGKGGVAYIMKTDHGLQIPRSMQVEFSTVVQNVTDAEGGEVNSKAMWDIFATEYLERTAPVEQIALRVENAQTENEDASITAELIHNGKDVTVDGRGNGPLAAYANALEKLGIDVEIQEYNQHAHTSDDDAEAAAYVLAEVNGRKVWGVGIAGSITYASLKAVTSAVNRALDVNHEAVLAGGV

SEQ ID NO: 41 - DNA, 1851 bp, Artificial Sequence
  H162E, P247C, R558H, G561D
atgtctcctaacgatgcattcatctccgcacctgccaagatcgaaaccccagttgggcctcgcaatgaaggccagccagcatggaataagcagcgtggctcctcaatgccagttaaccgctacatgcctttcgaggttgaggtagaagatatttctctgccggaccgcacttggccagataaaaaaatcaccgttgcacctcagtggtgtgctgttgacctgcgtgacggcaaccaggctctgattgatccgatgtctcctgagcgtaagcgccgcatgtttgagctgctggttcagatgggattcaaggaaatcgaggtcggtttcccttcagcttcccagactgattttgatttcgttcgtgagatcatcgaaaaggacatgatccctgacgatgtcaccattcaggttctggttcaggctcgtgagcacctgattcgccgtacttttgaagcttgcgaaggcgcaaaaaacgttatcgtggagttctacaactcaacctccatcctgcagcgcaacgtggtgttccgcatggacaaggtgcaggtgaagaagctggctaccgatgccgctgaactgatcaagaccgtcgctcaggattacccagacaccaactggcgctggcagtactcccctgagtccttcaccggcactgaggttgagtacgccaaggaagttgtggacgcagttgttgaggtcatggatccaactcctgagaacccaatgatcatcaacctgtgttccaccgttgagatgatcacccctaacgtttacgcagactccattgaatggatgcaccgcaatctaaaccgtcgtgattccattatcctgtccctgcacccgcacaatgaccgtggcaccggcgttggcgcagctgagctgggctacatggctggcgctgaccgcatcgaaggctgcctgttcggcaacggcgagcgcaccggcaacgtctgcctggtcaccctggcactgaacatgctgacccagggcgttgaccctcagctggacttcaccgatatacgccagatccgcagcaccgttgaatactgcaaccagctgcgcgttcctgagcgccacccatacggcggcgacctggtcttcaccgctttctccggttcccaccaggacgctgtgaacaagggtctggacgccatggctgccaaggttcagccaggtgctagctccactgaagtttcttgggagcagctgcgcgacaccgaatgggaggttccttacctgcctatcgatccaaaggatgtcggtcgcgactacgaggctgttatccgcgtgaactcccagtccggcaagggcggcgttgcttacatcatgaagaccgatcacggtctgcagatccctcgctccatgcaggttgagttctccaccgttgtccagaacgtcaccgacgctgagggcggcgaggtcaactccaaggcaatgtgggatatcttcgccaccgagtacctggagcgcaccgcaccagttgagcagatcgcgctgcgcgtcgagaacgctcagaccgaaaacgaggatgcatccatcaccgccgagctcatccacaacggcaaggacgtcaccgtcgatggccacggcaacggcccactggctgcttacgccaacgcgctggagaagctgggcatcgacgttgagatccaggaatacaaccagcacgcccacacctcggatgacgatgcagaagcagccgcctacgtgctggctgaggtcaacggccgcaaggtctggggcgtcggcatcgctggctccatcacctacgcttcgctgaaggcagtgacctccgccgtaaaccgcgcgctggacgtcaaccacgaggcagtcctggctggcggcgtttaa

SEQ ID NO: 42 - protein, 616 aa, Artificial Sequence
  S211L, P247C, R558H, G561D
MSPNDAFISAPAKIETPVGPRNEGQPAWNKQRGSSMPVNRYMPFEVEVEDISLPDRTWPDKKITVAPQWCAVDLRDGNQALIDPMSPERKRRMFELLVQMGFKEIEVGFPSASQTDFDFVREIIEKGMIPDDVTIQVLVQAREHLIRRTFEACEGAKNVIVHFYNSTSILQRNVVFRMDKVQVKKLATDAAELIKTIAQDYPDTNWRWQYLPESFTGTEVEYAKEVVDAVVEVMDPTPENPMIINLCSTVEMITPNVYADSIEWMHRNLNRRDSIILSLHPHNDRGTGVGAAELGYMAGADRIEGCLFGNGERTGNVCLVTLALNMLTQGVDPQLDFTDIRQIRSTVEYCNQLRVPERHPYGGDLVFTAFSGSHQDAVNKGLDAMAAKVQPGASSTEVSWEQLRDTEWEVPYLPIDPKDVGRDYEAVIRVNSQSGKGGVAYIMKTDHGLQIPRSMQVEFSTVVQNVTDAEGGEVNSKAMWDIFATEYLERTAPVEQIALRVENAQTENEDASITAELIHNGKDVTVDGRGNGPLAAYANALEKLGIDVEIQEYNQHAHTSDDDAEAAAYVLAEVNGRKVWGVGIAGSITYASLKAVTSAVNRALDVNHEAVLAGGV

SEQ ID NO: 43 - DNA, 1851 bp, Artificial Sequence
  S211L, P247C, R558H, G561D
atgtctcctaacgatgcattcatctccgcacctgccaagatcgaaaccccagttgggcctcgcaatgaaggccagccagcatggaataagcagcgtggctcctcaatgccagttaaccgctacatgcctttcgaggttgaggtagaagatatttctctgccggaccgcacttggccagataaaaaaatcaccgttgcacctcagtggtgtgctgttgacctgcgtgacggcaaccaggctctgattgatccgatgtctcctgagcgtaagcgccgcatgtttgagctgctggttcagatgggattcaaggaaatcgaggtcggtttcccttcagcttcccagactgattttgatttcgttcgtgagatcatcgaaaaggacatgatccctgacgatgtcaccattcaggttctggttcaggctcgtgagcacctgattcgccgtacttttgaagcttgcgaaggcgcaaaaaacgttatcgtgcacttctacaactcaacctccatcctgcagcgcaacgtggtgttccgcatggacaaggtgcaggtgaagaagctggctaccgatgccgctgaactgatcaagaccgtcgctcaggattacccagacaccaactggcgctggcagtaccttcctgagtccttcaccggcactgaggttgagtacgccaaggaagttgtggacgcagttgttgaggtcatggatccaactcctgagaacccaatgatcatcaacctgtgttccaccgttgagatgatcacccctaacgtttacgcagactccattgaatggatgcaccgcaatctaaaccgtcgtgattccattatcctgtccctgcacccgcacaatgaccgtggcaccggcgttggcgcagctgagctgggctacatggctggcgctgaccgcatcgaaggctgcctgttcggcaacggcgagcgcaccggcaacgtctgcctggtcaccctggcactgaacatgctgacccagggcgttgaccctcagctggacttcaccgatatacgccagatccgcagcaccgttgaatactgcaaccagctgcgcgttcctgagcgccacccatacggcggcgacctggtcttcaccgctttctccggttcccaccaggacgctgtgaacaagggtctggacgccatggctgccaaggttcagccaggtgctagctccactgaagtttcttgggagcagctgcgcgacaccgaatgggaggttccttacctgcctatcgatccaaaggatgtcggtcgcgactacgaggctgttatccgcgtgaactcccagtccggcaagggcggcgttgcttacatcatgaagaccgatcacggtctgcagatccctcgctccatgcaggttgagttctccaccgttgtccagaacgtcaccgacgctgagggcggcgaggtcaactccaaggcaatgtgggatatcttcgccaccgagtacctggagcgcaccgcaccagttgagcagatcgcgctgcgcgtcgagaacgctcagaccgaaaacgaggatgcatccatcaccgccgagctcatccacaacggcaaggacgtcaccgtcgatggccacggcaacggcccactggctgcttacgccaacgcgctggagaagctgggcatcgacgttgagatccaggaatacaaccagcacgcccacacctcggatgacgatgcagaagcagccgcctacgtgctggctgaggtcaacggccgcaaggtctggggcgtcggcatcgctggctccatcacctacgcttcgctgaaggcagtgacctccgccgtaaaccgcgcgctggacgtcaaccacgaggcagtcctggctggcggcgtttaa

SEQ ID NO: 44 - protein, 616 aa, Artificial Sequence
  N245S, P247C, R558H, G561D
MSPNDAFISAPAKIETPVGPRNEGQPAWNKQRGSSMPVNRYMPFEVEVEDISLPDRTWPDKKITVAPQWCAVDLRDGNQALIDPMSPERKRRMFELLVQMGFKEIEVGFPSASQTDFDFVREIIEKGMIPDDVTIQVLVQAREHLIRRTFEACEGAKNVIVHFYNSTSILQRNVVFRMDKVQVKKLATDAAELIKTIAQDYPDTNWRWQYSPESFTGTEVEYAKEVVDAVVEVMDPTPENPMIISLCSTVEMITPNVYADSIEWMHRNLNRRDSIILSLHPHNDRGTGVGAAELGYMAGADRIEGCLFGNGERTGNVCLVTLALNMLTQGVDPQLDFTDIRQIRSTVEYCNQLRVPERHPYGGDLVFTAFSGSHQDAVNKGLDAMAAKVQPGASSTEVSWEQLRDTEWEVPYLPIDPKDVGRDYEAVIRVNSQSGKGGVAYIMKTDHGLQIPRSMQVEFSTVVQNVTDAEGGEVNSKAMWDIFATEYLERTAPVEQIALRVENAQTENEDASITAELIHNGKDVTVDGRGNGPLAAYANALEKLGIDVEIQEYNQHAHTSDDDAEAAAYVLAEVNGRKVWGVGIAGSITYASLKAVTSAVNRALDVNHEAVLAGGV

SEQ ID NO: 45 - DNA, 1851 bp, Artificial Sequence
  N245S, P247C, R558H, G561D
atgtctcctaacgatgcattcatctccgcacctgccaagatcgaaaccccagttgggcctcgcaatgaaggccagccagcatggaataagcagcgtggctcctcaatgccagttaaccgctacatgcctttcgaggttgaggtagaagatatttctctgccggaccgcacttggccagataaaaaaatcaccgttgcacctcagtggtgtgctgttgacctgcgtgacggcaaccaggctctgattgatccgatgtctcctgagcgtaagcgccgcatgtttgagctgctggttcagatgggattcaaggaaatcgaggtcggtttcccttcagcttcccagactgattttgatttcgttcgtgagatcatcgaaaaggacatgatccctgacgatgtcaccattcaggttctggttcaggctcgtgagcacctgattcgccgtacttttgaagcttgcgaaggcgcaaaaaacgttatcgtgcacttctacaactcaacctccatcctgcagcgcaacgtggtgttccgcatggacaaggtgcaggtgaagaagctggctaccgatgccgctgaactgatcaagaccgtcgctcaggattacccagacaccaactggcgctggcagtactcccctgagtccttcaccggcactgaggttgagtacgccaaggaagttgtggacgcagttgttgaggtcatggatccaactcctgagaacccaatgatcatctccctgtgttccaccgttgagatgatcacccctaacgtttacgcagactccattgaatggatgcaccgcaatctaaaccgtcgtgattccattatcctgtccctgcacccgcacaatgaccgtggcaccggcgttggcgcagctgagctgggctacatggctggcgctgaccgcatcgaaggctgcctgttcggcaacggcgagcgcaccggcaacgtctgcctggtcaccctggcactgaacatgctgacccagggcgttgaccctcagctggacttcaccgatatacgccagatccgcagcaccgttgaatactgcaaccagctgcgcgttcctgagcgccacccatacggcggcgacctggtcttcaccgctttctccggttcccaccaggacgctgtgaacaagggtctggacgccatggctgccaaggttcagccaggtgctagctccactgaagtttcttgggagcagctgcgcgacaccgaatgggaggttccttacctgcctatcgatccaaaggatgtcggtcgcgactacgaggctgttatccgcgtgaactcccagtccggcaagggcggcgttgcttacatcatgaagaccgatcacggtctgcagatccctcgctccatgcaggttgagttctccaccgttgtccagaacgtcaccgacgctgagggcggcgaggtcaactccaaggcaatgtgggatatcttcgccaccgagtacctggagcgcaccgcaccagttgagcagatcgcgctgcgcgtcgagaacgctcagaccgaaaacgaggatgcatccatcaccgccgagctcatccacaacggcaaggacgtcaccgtcgatggccacggcaacggcccactggctgcttacgccaacgcgctggagaagctgggcatcgacgttgagatccaggaatacaaccagcacgcccacacctcggatgacgatgcagaagcagccgcctacgtgctggctgaggtcaacggccgcaaggtctggggcgtcggcatcgctggctccatcacctacgcttcgctgaaggcagtgacctccgccgtaaaccgcgcgctggacgtcaaccacgaggcagtcctggctggcggcgtttaa

SEQ ID NO: 46 - protein, 616 aa, Artificial Sequence
  I588P, P247C, R558H, G561D
MSPNDAFISAPAKIETPVGPRNEGQPAWNKQRGSSMPVNRYMPFEVEVEDISLPDRTWPDKKITVAPQWCAVDLRDGNQALIDPMSPERKRRMFELLVQMGFKEIEVGFPSASQTDFDFVREIIEKGMIPDDVTIQVLVQAREHLIRRTFEACEGAKNVIVHFYNSTSILQRNVVFRMDKVQVKKLATDAAELIKTIAQDYPDTNWRWQYSPESFTGTEVEYAKEVVDAVVEVMDPTPENPMIINLCSTVEMITPNVYADSIEWMHRNLNRRDSIILSLHPHNDRGTGVGAAELGYMAGADRIEGCLFGNGERTGNVCLVTLALNMLTQGVDPQLDFTDIRQIRSTVEYCNQLRVPERHPYGGDLVFTAFSGSHQDAVNKGLDAMAAKVQPGASSTEVSWEQLRDTEWEVPYLPIDPKDVGRDYEAVIRVNSQSGKGGVAYIMKTDHGLQIPRSMQVEFSTVVQNVTDAEGGEVNSKAMWDIFATEYLERTAPVEQIALRVENAQTENEDASITAELIHNGKDVTVDGRGNGPLAAYANALEKLGIDVEIQEYNQHAHTSDDDAEAAAYVLAEVNGRKVWGVGIAGSPTYASLKAVTSAVNRALDVNHEAVLAGGV

SEQ ID NO: 47 - DNA, 1851 bp, Artificial Sequence
  I588P, P247C, R558H, G561D
atgtctcctaacgatgcattcatctccgcacctgccaagatcgaaaccccagttgggcctcgcaatgaaggccagccagcatggaataagcagcgtggctcctcaatgccagttaaccgctacatgcctttcgaggttgaggtagaagatatttctctgccggaccgcacttggccagataaaaaaatcaccgttgcacctcagtggtgtgctgttgacctgcgtgacggcaaccaggctctgattgatccgatgtctcctgagcgtaagcgccgcatgtttgagctgctggttcagatgggattcaaggaaatcgaggtcggtttcccttcagcttcccagactgattttgatttcgttcgtgagatcatcgaaaaggacatgatccctgacgatgtcaccattcaggttctggttcaggctcgtgagcacctgattcgccgtacttttgaagcttgcgaaggcgcaaaaaacgttatcgtgcacttctacaactcaacctccatcctgcagcgcaacgtggtgttccgcatggacaaggtgcaggtgaagaagctggctaccgatgccgctgaactgatcaagaccgtcgctcaggattacccagacaccaactggcgctggcagtactcccctgagtccttcaccggcactgaggttgagtacgccaaggaagttgtggacgcagttgttgaggtcatggatccaactcctgagaacccaatgatcatcaacctgtgttccaccgttgagatgatcacccctaacgtttacgcagactccattgaatggatgcaccgcaatctaaaccgtcgtgattccattatcctgtccctgcacccgcacaatgaccgtggcaccggcgttggcgcagctgagctgggctacatggctggcgctgaccgcatcgaaggctgcctgttcggcaacggcgagcgcaccggcaacgtctgcctggtcaccctggcactgaacatgctgacccagggcgttgaccctcagctggacttcaccgatatacgccagatccgcagcaccgttgaatactgcaaccagctgcgcgttcctgagcgccacccatacggcggcgacctggtcttcaccgctttctccggttcccaccaggacgctgtgaacaagggtctggacgccatggctgccaaggttcagccaggtgctagctccactgaagtttcttgggagcagctgcgcgacaccgaatgggaggttccttacctgcctatcgatccaaaggatgtcggtcgcgactacgaggctgttatccgcgtgaactcccagtccggcaagggcggcgttgcttacatcatgaagaccgatcacggtctgcagatccctcgctccatgcaggttgagttctccaccgttgtccagaacgtcaccgacgctgagggcggcgaggtcaactccaaggcaatgtgggatatcttcgccaccgagtacctggagcgcaccgcaccagttgagcagatcgcgctgcgcgtcgagaacgctcagaccgaaaacgaggatgcatccatcaccgccgagctcatccacaacggcaaggacgtcaccgtcgatggccacggcaacggcccactggctgcttacgccaacgcgctggagaagctgggcatcgacgttgagatccaggaatacaaccagcacgcccacacctcggatgacgatgcagaagcagccgcctacgtgctggctgaggtcaacggccgcaaggtctggggcgtcggcatcgctggctcccccacctacgcttcgctgaaggcagtgacctccgccgtaaaccgcgcgctggacgtcaaccacgaggcagtcctggctggcggcgtttaa

SEQ ID NO: 48 - protein, 616 aa, Artificial Sequence
  S211L,  P247C, R558H, G561D, I588P
MSPNDAFISAPAKIETPVGPRNEGQPAWNKQRGSSMPVNRYMPFEVEVEDISLPDRTWPDKKITVAPQWCAVDLRDGNQALIDPMSPERKRRMFELLVQMGFKEIEVGFPSASQTDFDFVREIIEKGMIPDDVTIQVLVQAREHLIRRTFEACEGAKNVIVHFYNSTSILQRNVVFRMDKVQVKKLATDAAELIKTIAQDYPDTNWRWQYLPESFTGTEVEYAKEVVDAVVEVMDPTPENPMIINLCSTVEMITPNVYADSIEWMHRNLNRRDSIILSLHPHNDRGTGVGAAELGYMAGADRIEGCLFGNGERTGNVCLVTLALNMLTQGVDPQLDFTDIRQIRSTVEYCNQLRVPERHPYGGDLVFTAFSGSHQDAVNKGLDAMAAKVQPGASSTEVSWEQLRDTEWEVPYLPIDPKDVGRDYEAVIRVNSQSGKGGVAYIMKTDHGLQIPRSMQVEFSTVVQNVTDAEGGEVNSKAMWDIFATEYLERTAPVEQIALRVENAQTENEDASITAELIHNGKDVTVDGRGNGPLAAYANALEKLGIDVEIQEYNQHAHTSDDDAEAAAYVLAEVNGRKVWGVGIAGSPTYASLKAVTSAVNRALDVNHEAVLAGGV

SEQ ID NO: 49 - DNA, 1851 bp, Artificial Sequence
  S211L,  P247C, R558H, G561D, I588P
atgtctcctaacgatgcattcatctccgcacctgccaagatcgaaaccccagttgggcctcgcaatgaaggccagccagcatggaataagcagcgtggctcctcaatgccagttaaccgctacatgcctttcgaggttgaggtagaagatatttctctgccggaccgcacttggccagataaaaaaatcaccgttgcacctcagtggtgtgctgttgacctgcgtgacggcaaccaggctctgattgatccgatgtctcctgagcgtaagcgccgcatgtttgagctgctggttcagatgggattcaaggaaatcgaggtcggtttcccttcagcttcccagactgattttgatttcgttcgtgagatcatcgaaaaggacatgatccctgacgatgtcaccattcaggttctggttcaggctcgtgagcacctgattcgccgtacttttgaagcttgcgaaggcgcaaaaaacgttatcgtgcacttctacaactcaacctccatcctgcagcgcaacgtggtgttccgcatggacaaggtgcaggtgaagaagctggctaccgatgccgctgaactgatcaagaccgtcgctcaggattacccagacaccaactggcgctggcagtaccttcctgagtccttcaccggcactgaggttgagtacgccaaggaagttgtggacgcagttgttgaggtcatggatccaactcctgagaacccaatgatcatcaacctgtgttccaccgttgagatgatcacccctaacgtttacgcagactccattgaatggatgcaccgcaatctaaaccgtcgtgattccattatcctgtccctgcacccgcacaatgaccgtggcaccggcgttggcgcagctgagctgggctacatggctggcgctgaccgcatcgaaggctgcctgttcggcaacggcgagcgcaccggcaacgtctgcctggtcaccctggcactgaacatgctgacccagggcgttgaccctcagctggacttcaccgatatacgccagatccgcagcaccgttgaatactgcaaccagctgcgcgttcctgagcgccacccatacggcggcgacctggtcttcaccgctttctccggttcccaccaggacgctgtgaacaagggtctggacgccatggctgccaaggttcagccaggtgctagctccactgaagtttcttgggagcagctgcgcgacaccgaatgggaggttccttacctgcctatcgatccaaaggatgtcggtcgcgactacgaggctgttatccgcgtgaactcccagtccggcaagggcggcgttgcttacatcatgaagaccgatcacggtctgcagatccctcgctccatgcaggttgagttctccaccgttgtccagaacgtcaccgacgctgagggcggcgaggtcaactccaaggcaatgtgggatatcttcgccaccgagtacctggagcgcaccgcaccagttgagcagatcgcgctgcgcgtcgagaacgctcagaccgaaaacgaggatgcatccatcaccgccgagctcatccacaacggcaaggacgtcaccgtcgatggccacggcaacggcccactggctgcttacgccaacgcgctggagaagctgggcatcgacgttgagatccaggaatacaaccagcacgcccacacctcggatgacgatgcagaagcagccgcctacgtgctggctgaggtcaacggccgcaaggtctggggcgtcggcatcgctggctcccccacctacgcttcgctgaaggcagtgacctccgccgtaaaccgcgcgctggacgtcaaccacgaggcagtcctggctggcggcgtttaa

SEQ ID NO: 50 - protein, 616 aa, Artificial Sequence
  L138G, H162E, S211L, N245S, P247C, R558H, G561D
MSPNDAFISAPAKIETPVGPRNEGQPAWNKQRGSSMPVNRYMPFEVEVEDISLPDRTWPDKKITVAPQWCAVDLRDGNQALIDPMSPERKRRMFELLVQMGFKEIEVGFPSASQTDFDFVREIIEKGMIPDDVTIQVGVQAREHLIRRTFEACEGAKNVIVEFYNSTSILQRNVVFRMDKVQVKKLATDAAELIKTIAQDYPDTNWRWQYLPESFTGTEVEYAKEVVDAVVEVMDPTPENPMIISLCSTVEMITPNVYADSIEWMHRNLNRRDSIILSLHPHNDRGTGVGAAELGYMAGADRIEGCLFGNGERTGNVCLVTLALNMLTQGVDPQLDFTDIRQIRSTVEYCNQLRVPERHPYGGDLVFTAFSGSHQDAVNKGLDAMAAKVQPGASSTEVSWEQLRDTEWEVPYLPIDPKDVGRDYEAVIRVNSQSGKGGVAYIMKTDHGLQIPRSMQVEFSTVVQNVTDAEGGEVNSKAMWDIFATEYLERTAPVEQIALRVENAQTENEDASITAELIHNGKDVTVDGRGNGPLAAYANALEKLGIDVEIQEYNQHAHTSDDDAEAAAYVLAEVNGRKVWGVGIAGSITYASLKAVTSAVNRALDVNHEAVLAGGV

SEQ ID NO: 51 - DNA, 1851 bp, Artificial Sequence
  L138G, H162E, S211L, N245S, P247C, R558H, G561D
atgtctcctaacgatgcattcatctccgcacctgccaagatcgaaaccccagttgggcctcgcaatgaaggccagccagcatggaataagcagcgtggctcctcaatgccagttaaccgctacatgcctttcgaggttgaggtagaagatatttctctgccggaccgcacttggccagataaaaaaatcaccgttgcacctcagtggtgtgctgttgacctgcgtgacggcaaccaggctctgattgatccgatgtctcctgagcgtaagcgccgcatgtttgagctgctggttcagatgggattcaaggaaatcgaggtcggtttcccttcagcttcccagactgattttgatttcgttcgtgagatcatcgaaaaggacatgatccctgacgatgtcaccattcaggttggggttcaggctcgtgagcacctgattcgccgtacttttgaagcttgcgaaggcgcaaaaaacgttatcgtggagttctacaactcaacctccatcctgcagcgcaacgtggtgttccgcatggacaaggtgcaggtgaagaagctggctaccgatgccgctgaactgatcaagaccgtcgctcaggattacccagacaccaactggcgctggcagtaccttcctgagtccttcaccggcactgaggttgagtacgccaaggaagttgtggacgcagttgttgaggtcatggatccaactcctgagaacccaatgatcatctccctgtgttccaccgttgagatgatcacccctaacgtttacgcagactccattgaatggatgcaccgcaatctaaaccgtcgtgattccattatcctgtccctgcacccgcacaatgaccgtggcaccggcgttggcgcagctgagctgggctacatggctggcgctgaccgcatcgaaggctgcctgttcggcaacggcgagcgcaccggcaacgtctgcctggtcaccctggcactgaacatgctgacccagggcgttgaccctcagctggacttcaccgatatacgccagatccgcagcaccgttgaatactgcaaccagctgcgcgttcctgagcgccacccatacggcggcgacctggtcttcaccgctttctccggttcccaccaggacgctgtgaacaagggtctggacgccatggctgccaaggttcagccaggtgctagctccactgaagtttcttgggagcagctgcgcgacaccgaatgggaggttccttacctgcctatcgatccaaaggatgtcggtcgcgactacgaggctgttatccgcgtgaactcccagtccggcaagggcggcgttgcttacatcatgaagaccgatcacggtctgcagatccctcgctccatgcaggttgagttctccaccgttgtccagaacgtcaccgacgctgagggcggcgaggtcaactccaaggcaatgtgggatatcttcgccaccgagtacctggagcgcaccgcaccagttgagcagatcgcgctgcgcgtcgagaacgctcagaccgaaaacgaggatgcatccatcaccgccgagctcatccacaacggcaaggacgtcaccgtcgatggccacggcaacggcccactggctgcttacgccaacgcgctggagaagctgggcatcgacgttgagatccaggaatacaaccagcacgcccacacctcggatgacgatgcagaagcagccgcctacgtgctggctgaggtcaacggccgcaaggtctggggcgtcggcatcgctggctccatcacctacgcttcgctgaaggcagtgacctccgccgtaaaccgcgcgctggacgtcaaccacgaggcagtcctggctggcggcgtttaa

SEQ ID NO: 52 - protein, 616 aa, Artificial Sequence
  L138G, H162E, S211L, N245S, P247C, R558H, G561D, I588P
MSPNDAFISAPAKIETPVGPRNEGQPAWNKQRGSSMPVNRYMPFEVEVEDISLPDRTWPDKKITVAPQWCAVDLRDGNQALIDPMSPERKRRMFELLVQMGFKEIEVGFPSASQTDFDFVREIIEKGMIPDDVTIQVGVQAREHLIRRTFEACEGAKNVIVEFYNSTSILQRNVVFRMDKVQVKKLATDAAELIKTIAQDYPDTNWRWQYLPESFTGTEVEYAKEVVDAVVEVMDPTPENPMIISLCSTVEMITPNVYADSIEWMHRNLNRRDSIILSLHPHNDRGTGVGAAELGYMAGADRIEGCLFGNGERTGNVCLVTLALNMLTQGVDPQLDFTDIRQIRSTVEYCNQLRVPERHPYGGDLVFTAFSGSHQDAVNKGLDAMAAKVQPGASSTEVSWEQLRDTEWEVPYLPIDPKDVGRDYEAVIRVNSQSGKGGVAYIMKTDHGLQIPRSMQVEFSTVVQNVTDAEGGEVNSKAMWDIFATEYLERTAPVEQIALRVENAQTENEDASITAELIHNGKDVTVDGRGNGPLAAYANALEKLGIDVEIQEYNQHAHTSDDDAEAAAYVLAEVNGRKVWGVGIAGSPTYASLKAVTSAVNRALDVNHEAVLAGGV

SEQ ID NO: 53 - DNA, 1851 bp, Artificial Sequence
  L138G, H162E, S211L, N245S, P247C, R558H, G561D, I588P
atgtctcctaacgatgcattcatctccgcacctgccaagatcgaaaccccagttgggcctcgcaatgaaggccagccagcatggaataagcagcgtggctcctcaatgccagttaaccgctacatgcctttcgaggttgaggtagaagatatttctctgccggaccgcacttggccagataaaaaaatcaccgttgcacctcagtggtgtgctgttgacctgcgtgacggcaaccaggctctgattgatccgatgtctcctgagcgtaagcgccgcatgtttgagctgctggttcagatgggattcaaggaaatcgaggtcggtttcccttcagcttcccagactgattttgatttcgttcgtgagatcatcgaaaaggacatgatccctgacgatgtcaccattcaggttggggttcaggctcgtgagcacctgattcgccgtacttttgaagcttgcgaaggcgcaaaaaacgttatcgtggagttctacaactcaacctccatcctgcagcgcaacgtggtgttccgcatggacaaggtgcaggtgaagaagctggctaccgatgccgctgaactgatcaagaccgtcgctcaggattacccagacaccaactggcgctggcagtaccttcctgagtccttcaccggcactgaggttgagtacgccaaggaagttgtggacgcagttgttgaggtcatggatccaactcctgagaacccaatgatcatctccctgtgttccaccgttgagatgatcacccctaacgtttacgcagactccattgaatggatgcaccgcaatctaaaccgtcgtgattccattatcctgtccctgcacccgcacaatgaccgtggcaccggcgttggcgcagctgagctgggctacatggctggcgctgaccgcatcgaaggctgcctgttcggcaacggcgagcgcaccggcaacgtctgcctggtcaccctggcactgaacatgctgacccagggcgttgaccctcagctggacttcaccgatatacgccagatccgcagcaccgttgaatactgcaaccagctgcgcgttcctgagcgccacccatacggcggcgacctggtcttcaccgctttctccggttcccaccaggacgctgtgaacaagggtctggacgccatggctgccaaggttcagccaggtgctagctccactgaagtttcttgggagcagctgcgcgacaccgaatgggaggttccttacctgcctatcgatccaaaggatgtcggtcgcgactacgaggctgttatccgcgtgaactcccagtccggcaagggcggcgttgcttacatcatgaagaccgatcacggtctgcagatccctcgctccatgcaggttgagttctccaccgttgtccagaacgtcaccgacgctgagggcggcgaggtcaactccaaggcaatgtgggatatcttcgccaccgagtacctggagcgcaccgcaccagttgagcagatcgcgctgcgcgtcgagaacgctcagaccgaaaacgaggatgcatccatcaccgccgagctcatccacaacggcaaggacgtcaccgtcgatggccacggcaacggcccactggctgcttacgccaacgcgctggagaagctgggcatcgacgttgagatccaggaatacaaccagcacgcccacacctcggatgacgatgcagaagcagccgcctacgtgctggctgaggtcaacggccgcaaggtctggggcgtcggcatcgctggctcccccacctacgcttcgctgaaggcagtgacctccgccgtaaaccgcgcgctggacgtcaaccacgaggcagtcctggctggcggcgtttaa

SEQ ID NO: 54 - DNA, 45 bp, Artificial Sequence
  Primer 27
ggtgatcatctcaacggtggaacacaggttgatgatcattgggtt

SEQ ID NO: 55 - DNA, 45 bp, Artificial Sequence
  Primer 28
aacccaatgatcatcaacctgtgttccaccgttgagatgatcacc